European Patent Specification EP 3 320 099 B1, published September 13, 2023. Title: Lentiviral vector expressing membrane-anchored or secreted antibody. Applicant: INSERM Université Claude Bernard Lyon 1 CNRS Ecole normale supérieure de Lyon. The sequence listing filed with the application follows.

SEQUENCE LISTING (32 sequences)

SEQ ID NO: 1 - protein, 8 aa, Artificial Sequence
  2A peptides consensus motif
  misc_feature (2)..(2): Xaa can be any naturally occurring amino acid
  misc_feature (4)..(4): Xaa can be any naturally occurring amino acid
DXEXNPGP

SEQ ID NO: 2 - protein, 22 aa, Foot-and-mouth disease virus
VKQTLNFDLLKLAGDVESNPGP

SEQ ID NO: 3 - DNA, 66 bp, Foot-and-mouth disease virus
gtgaaacagactttgaattttgaccttctcaagttggcaggagacgttgagtccaaccctgggccc

SEQ ID NO: 4 - protein, 18 aa, Artificial Sequence
  T2A peptide
EGRGSLLTCGDVEENPGP

SEQ ID NO: 5 - DNA, 51 bp, Artificial Sequence
  sequence encoding T2A peptide
ggcaggggaagtcttctaacatgcggggacgtggaggaaaatcccggcccc

SEQ ID NO: 6 - protein, 19 aa, Artificial Sequence
  P2A peptide
ATNFSLLKQAGDVEENPGP

SEQ ID NO: 7 - DNA, 57 bp, Artificial Sequence
  sequence encoding P2A peptide
gccacaaacttttctttactaaaacaagcgggagatgttgaggaaaaccccgggcct

SEQ ID NO: 8 - protein, 20 aa, Artificial Sequence
  E2A peptide
QCTNYALLKLAGDVESNPGP

SEQ ID NO: 9 - DNA, 60 bp, Artificial Sequence
  sequence encoding E2A peptide
cagtgtactaactatgctttgttgaaattagctggggatgttgagagcaaccccggccct

SEQ ID NO: 10 - DNA, 66 bp, Artificial Sequence
  codon optimized sequence encoding F2A peptide
gtgaaacagactttgaattttgaccttctcaagttggcgggagacgtggagtccaacccagggccc

SEQ ID NO: 11 - DNA, 54 bp, Artificial Sequence
  codon optimized sequence encoding T2A peptide
gagggcagaggaagtctgctaacatgcggtgacgtcgaggagaatcctggccca

SEQ ID NO: 12 - DNA, 60 bp, Artificial Sequence
  codon optimized sequence encoding E2A peptide
caatgtactaactacgctttgttgaaactcgctggcgatgttgaaagtaaccccggtcct

SEQ ID NO: 13 - protein, 5 aa, Artificial Sequence
  furin cleavage site consensus sequence
  misc_feature (2)..(2): Xaa can be any naturally occurring amino acid
RXKRR

SEQ ID NO: 14 - protein, 4 aa, Artificial Sequence
  furin cleavage site
RAKR

SEQ ID NO: 15 - DNA, 12 bp, Artificial Sequence
  sequence encoding a furin cleavage site
cgggctaagaga

SEQ ID NO: 16 - DNA, 1272 bp, Artificial Sequence
  MH promoter
ggattgtttatcttaggaggcatgcttactgttaaaagacaggatatgtttgaagtggcttctgagaaaaatggttaagaaaattatgacttaaaaatgtgagagattttcaagtatattaatttttttaactgtccaagtatttgaaattcttatcatttgattaacacccatgagtgatatgtgtctggaattgaggccaaagcaagctcagctaagaaatactagcacagtgctgtcggccccgatgcgggactgcgttttgaccatcataaatcaagtttatttttttaattaattgagcgaagctggaagcagatgatgaattagagtcaagatggctgcatgggggtctccggcacccacagcaggtggcaggaagcaggtcaccgcgagagtctattttaggaagcaaaaaaacacaattggtaaatttatcacttctggttgtgaagaggtggttttgcccaggcccagatctgaaagtgctctactgagcaaaacaacacctggacaatttgcgtttctaaaataaggcgaggctgaccgaaactgaaaaggctttttttaactatctgaatttcatttccaatcttagcttatcaactgctagtttgtgcaaacagcatatcaacttctaaactgcattcatttttaaagtaagatgtttaagaaattaaacagtcttagggagagtttatgactgtattcaaaaagttttttaaattagcttgttatcccttcatgtgataactaatctcaaatactttttcgatacctcagagcattattttcataatgactgtgttcacaatctttttaggttaactcgttttctctttgtgattaaggagaaacactttgatattctgatagagtggccttcattttagtatttttcaagaccacttttcaactactcactttaggataagttttaggtaaaatgtgcatcattatcctgaattatttcagttaagcatgttagttggtggcataagagaaaactcaatcagataggtaccgcgggcccgggatccgcaggatttagggcttggtctctcagcatcccacacttgtacagctgatgtggcatctgtgttttctttctcatcctagatcaggctttgagctgtgaaataccctgcctcatgcatatgcaaataacctgaggtcttctgagataaatatagatatattggtgccctgagagcatcacataacaaccacattcctcctctgaagaagcccctgggagcacagctcatcacc

SEQ ID NO: 17 - DNA, 904 bp, Artificial Sequence
  FEEK promoter
taaaccggtgagtttcatggttacttgcctgagaagattaaaaaaagtaatgctaccttatgagggagagtcccagggaccaagatagcaactgtcatagcaaccgtcacactgctttggtcaaggagaagaccctttggggaactgaaaacagaaccttgagcacatctgttgctttcgctcccatcctcctccaacagggctgggtggagcactccacaccctttcaccggtcgtacggctcagccagagtaaaaatcacacccatgacctggccactgagggcttgatcaattcactttgaatttggcattaaataccattaaggtatattaactgattttaaaataagatatattcgtgaccatgtttttaactttcaaaaatgtagctgccagtgtgtgattttatttcagttgtacaaaatatctaaacctatagcaatgtgattaataaaaacttaaacatattttccagtaccttaattctgtgataggaaaattttaatctgagtattttaatttcataatctctaaaatagtttaatgatttgtcattgtgttgctgtcgtttaccccagctgatctcaaaagtgatatttaaggagattattttggtctgcaacaacttgatagggctcagcctctcccacccaacgggtggaatcccccagagggggatttccaagaggccacctggcagttgctgagggtcagaagtgaagctagccacttcctcttaggcaggtggccaagattacagttgacccgtacgtgcagctgtgcccagcctgccccatcccctgctcatttgcatgttcccagagcacaacctcctgccctgaagccttattaataggctggtcacactttgtgcaggagtcagactcagtcaggacacagct

SEQ ID NO: 18 - DNA, 153 bp, Artificial Sequence
  pAM signal
aataaatatctttattttcattacatctgtgtgttggttttttgtgtgaatcgatagtactaacatacgctctccatcaaaacaaaacgaaacaaaacaaactagcaaaataggctgtccccagtgcaagtgcaggtgccagaacatttctct

SEQ ID NO: 19 - DNA, 205 bp, Artificial Sequence
  RRE
tccttgggttcttgggagcagcaggaagcactatgggcgcagcgtcaatgacgctgacggtacaggccagacaattattgtctggtatagtgcagcagcagaacaatttgctgagggctattgaggcgcaacagcatctgttgcaactcacagtctggggcatcaagcagctccaggcaagaatcctggctgtggaaagatacct

SEQ ID NO: 20 - DNA, 125 bp, Artificial Sequence
  cPPT
tccacaattttaaaagaaaaggggggattggggggtacagtgcaggggaaagaatagtagacataatagcaacagacatacaaactaaagaattacaaaaacaaattacaaaaattcaaaatttt

SEQ ID NO: 21 - DNA, 589 bp, Artificial Sequence
  WPRE
aatcaacctctggattacaaaatttgtgaaagattgactggtattcttaactatgttgctccttttacgctatgtggatacgctgctttaatgcctttgtatcatgctattgcttcccgtatggctttcattttctcctccttgtataaatcctggttgctgtctctttatgaggagttgtggcccgttgtcaggcaacgtggcgtggtgtgcactgtgtttgctgacgcaacccccactggttggggcattgccaccacctgtcagctcctttccgggactttcgctttccccctccctattgccacggcggaactcatcgccgcctgccttgcccgctgctggacaggggctcggctgttgggcactgacaattccgtggtgttgtcggggaagctgacgtcctttccatggctgctcgcctgtgttgccacctggattctgcgcgggacgtccttctgctacgtcccttcggccctcaatccagcggaccttccttcccgcggcctgctgccggctctgcggcctcttccgcgtcttcgccttcgccctcagacgagtcggatctccctttgggccgcctccccgc

SEQ ID NO: 22 - DNA, 594 bp, Artificial Sequence
  optimized WPRE
aatcaacctctggattacaaaatttgtgaaagattgactggtattcttaactatgttgctccttttacgctatgtggatacgctgctttaatgcctttgtatcatgctattgcttcccgtatggctttcattttctcctccttgtataaatcctggttgctgtctctttatgaggagttgtggcccgttgtcaggcaacgtggcgtggtgtgcactgtgtttgctgacgcaacccccactggttggggcattgccaccacctgtcagctcctttccgggactttcgctttccccctccctattgccacggcggaactcatcgccgcctgccttgcccgctgctggacaggggctcggctgttgggcactgacaattccgtggtgttgtcggggaaatcatcgtcctttccttggctgctcgcctgtgttgccacctgcattctgcgcgggacgtccttctgctacgtcccttcggccctcaatccagcggaccttccttcccgcggcctgctgccggctctgcggcctcttccgcgtcttcgccttcgccctcagacgagtcggatctccctttgggccgcctccccgcatcga

SEQ ID NO: 23 - protein, 546 aa, Artificial Sequence
  modified BaEV envelope glycoprotein
MGFTTKIIFLYNLVLVYAGFDDPRKAIELVQKRYGRPCDCSGGQVSEPPSDRVSQVTCSGKTAYLMPDQRWKCKSIPKDTSPSGPLQECPCNSYQSSVHSSCYTSYQQCRSGNKTYYTATLLKTQTGGTSDVQVLGSTNKLIQSPCNGIKGQSICWSTTAPIHVSDGGGPLDTTRIKSVQRKLEEIHKALYPELQYHPLAIPKVRDNLMVDAQTLNILNATYNLLLMSNTSLVDDCWLCLKLGPPTPLAIPNFLLSYVTRSSDNISCLIIPPLLVQPMQFSNSSCLFSPSYNSTEEIDLGHVAFSNCTSITNVTGPICAVNGSVFLCGNNMAYTYLPTNWTGLCVLATLLPDIDIIPGDEPVPIPAIDHFIYRPKRAIQFIPLLAGLGITAAFTTGATGLGVSVTQYTKLSNQLISDVQILSSTIQDLQDQVDSLAEVVLQNRRGLDLLTAEQGGICLALQEKCCFYVNKSGIVRDKIKTLQEELERRRKDLASNPLWTGLQGLLPYLLPFLGPLLTLLLLLTIGPCIFNRLTAFINDKLNIIHAM

SEQ ID NO: 24 - DNA, 84 bp, Artificial Sequence
  F2A/furin peptide sequence
cgggctaagagagcaccggtgaaacagactttgaattttgaccttctcaagttggcgggagacgtggagtccaacccagggccc

SEQ ID NO: 25 - DNA, 20 bp, Artificial Sequence
  F primer
tgtgtgcccgtctgttgtgt

SEQ ID NO: 26 - DNA, 20 bp, Artificial Sequence
  R primer
gagtcctgcgtcgagagagc

SEQ ID NO: 27 - DNA, 20 bp, Artificial Sequence
  probe
cagtggcgcccgaacaggga

SEQ ID NO: 28 - DNA, 22 bp, Artificial Sequence
  actin F primer
tccgtgtggatcggcggctcca

SEQ ID NO: 29 - DNA, 21 bp, Artificial Sequence
  actin R primer
ctgcttgctgatccacatctg

SEQ ID NO: 30 - DNA, 24 bp, Artificial Sequence
  actin probe
cctggcctcgctgtccaccttcca

SEQ ID NO: 31 - DNA, 375 bp, Artificial Sequence
  typical B3 sequence
tgagtgccacggccggcaagcccccgctccccaggctctcggggtcgcgcgaggatgcttggcacgtaccccgtgtacatacttcccaggcacccagcatggaaataaagcacccagcgcttccctgggcccctgcgagactgtgatggttctttccacgggtcaggccgagtctgaggcctgagtggcatgagggaggcagagtgggtcccactgtccccacactggcccaggctgtggtggggagctgacctcaggacattgttggcccatcccggccgggccctacatcctgggtcctgccacagagggaatcacccccagaggcccaagcccagggggacacagcactgaccacccccttcctgtccagag

SEQ ID NO: 32 - DNA, 217 bp, Artificial Sequence
  typical B4 sequence
gtcggccgcacgttgtccccagctgtccttgacattgtcccccatgctgtcacaaactgtctctgacactgtcccacaggctgtccccacctgtccctgacgctgcgggtgggtgggccttgggggcagagaggtggcctcagtgccctgaggggtgggtggggctcgggggcagggctgtggcctcgctcacccctgtgctgtgccttgcctacag